European Patent Application EP 4 428 533 A1, published September 11, 2024. Title: 標的物質の検出方法. Applicant: 凸版印刷株式会社. Application WO. The sequence listing filed with the application follows.

SEQUENCE LISTING (7 sequences)

SEQ ID NO: 1 - DNA, 51 bp, synthetic construct
  misc_feature 1..51: note = Synthesized oligonucleotide
  source 1..51: mol_type = other DNA
tttgtcactgttcctccttttgttttcctttctgtgagcaatttcacccaa

SEQ ID NO: 2 - DNA, 22 bp, synthetic construct
  misc_feature 1..22: note = Synthesized oligonucleotide
  source 1..22: mol_type = other DNA
gcatggttccaatttgggtgat

SEQ ID NO: 3 - DNA, 28 bp, synthetic construct
  misc_feature 1..28: note = Synthesized oligonucleotide
  source 1..28: mol_type = other DNA
cgcgccgaggaattgctcacagaaagga

SEQ ID NO: 4 - DNA, 35 bp, synthetic construct
  misc_feature 1..35: note = Synthesized oligonucleotide
  misc_feature 1: note = Alexa488-amino-C6-modified nucleotide
  misc_feature 5: note = BHQ1-modified nucleotide
  source 1..35: mol_type = other DNA
ttcttagccggttttccggctgagacctcggcgcg

SEQ ID NO: 5 - DNA, 45 bp, synthetic construct
  source 1..45: mol_type = other DNA
tttgtcactgttcctccttttgttttcctttctgtgagcaatttc

SEQ ID NO: 6 - DNA, 54 bp, synthetic construct
  source 1..54: mol_type = other DNA
tttgtcactgttcctccttttgttttcctttctgtgagcaatttcacccaaatt

SEQ ID NO: 7 - DNA, 57 bp, synthetic construct
  source 1..57: mol_type = other DNA
tttgtcactgttcctccttttgttttcctttctgtgagcaatttcacccaaattgga